European Patent Application EP 4 316 588 A2, published February 7, 2024. Title: TREATMENT OF PRIMARY CILIARY DYSKINESIA WITH SYNTHETIC MESSENGER RNA. Applicant: Transcriptx, Inc. The sequence listing filed with the application follows.

SEQUENCE LISTING (20 sequences)

SEQ ID NO: 1 - DNA, 72 bp, synthetic construct
  misc_feature 1..72: note = Description of Artificial Sequence: Synthetic oligonucleotide
  source 1..72: mol_type = other DNA
gggagacataaaccctggcgcgctcgcggcccggcactcttctggtccccacagactcagagagaagccacc

SEQ ID NO: 2 - DNA, 72 bp, synthetic construct
  misc_feature 1..72: note = Description of Artificial Sequence: Synthetic oligonucleotide
  source 1..72: mol_type = other DNA
gggagacataaaccctggcgcgctcgcgggccggcactcttctggtccccacagactcagagagaagccacc

SEQ ID NO: 3 - DNA, 43 bp, synthetic construct
  misc_feature 1..43: note = Description of Artificial Sequence: Synthetic oligonucleotide
  source 1..43: mol_type = other DNA
gggagactcttctggtccccacagactcagagagaacgccacc

SEQ ID NO: 4 - DNA, 511 bp, synthetic construct
  misc_feature 1..511: note = Description of Artificial Sequence: Synthetic polynucleotide
  source 1..511: mol_type = other DNA
gttattttccaccatattgccgtcttttggcaatgtgagggcccggaaacctggccctgtcttcttgacgagcattcctaggggtctttcccctctcgccaaaggaatgcaaggtctgttgaatgtcgtgaaggaagcagttcctctggaagcttcttgaagacaaacaacgtctgtagcgaccctttgcaggcagcggaaccccccacctggcgacaggtgcctctgcggccaaaagccacgtgtataagatacacctgcaaaggcggcacaaccccagtgccacgttgtgagttggatagttgtggaaagagtcaaatggctctcctcaagcgtattcaacaaggggctgaaggatgcccagaaggtaccccattgtatgggatctgatctggggcctcggtgcacatgctttacgtgtgtttagtcgaggttaaaaaacgtctaggccccccgaaccacggggacgtggttttcctttgaaaaacacgatgataatatggccacaacc

SEQ ID NO: 5 - DNA, 143 bp, synthetic construct
  misc_feature 1..143: note = Description of Artificial Sequence: Synthetic polynucleotide
  source 1..143: mol_type = other DNA
aaataacaaatctcaacacaacatatacaaaacaaacgaatctcaagcaatcaagcattctacttctattgcagcaatttaaatcatttcttttaaagcaaaagcaattttctgaaaattttcaccatttacgaacgatagca

SEQ ID NO: 6 - DNA, 47 bp, synthetic construct
  misc_feature 1..47: note = Description of Artificial Sequence: Synthetic oligonucleotide
  source 1..47: mol_type = other DNA
gggagacaagagagaaaagaagagcaagaagaaatataagagccacc

SEQ ID NO: 7 - DNA, 66 bp, synthetic construct
  misc_feature 1..66: note = Description of Artificial Sequence: Synthetic oligonucleotide
  source 1..66: mol_type = other DNA
gggagacccaagctggctagcgtttaaacttaagcttggcaatccggtactgttggtaaagccacc

SEQ ID NO: 8 - DNA, 291 bp, synthetic construct
  misc_feature 1..291: note = Description of Artificial Sequence: Synthetic polynucleotide
  source 1..291: mol_type = other DNA
gggagacccaagctggctagcgtttaaacttaagctttcctttccgggccggctgggcgcgccgaagcgcctgcgccttggctgctggtcggttgctgggtaaccgcgtcagggagttggattctatcctgcaagggcacggggacccacaacgacggctgtccctaaagaaccgttgcgactggtaactgaagtggaagagagtccagatttcttgtgtgtggtcaaggagacggacaaactttttgtcttcagacgagggagcgttttgtaggctctccaggggttgag

SEQ ID NO: 9 - DNA, 186 bp, synthetic construct
  misc_feature 1..186: note = Description of Artificial Sequence: Synthetic polynucleotide
  source 1..186: mol_type = other DNA
ggattgtgtccgtaatcacacgtggtgcgtacgataacgcatagtgtttttccctccacttaaatcgaagggttgtgtcttggatcgcgcgggtcaaatgtatatggttcatatacatccgcaggcacgtaataaagcgaggggttcgaatccccccgttacccccggtaggggcccattgtcttc

SEQ ID NO: 10 - DNA, 114 bp, synthetic construct
  misc_feature 1..114: note = Description of Artificial Sequence: Synthetic polynucleotide
  source 1..114: mol_type = other DNA
tcagtagggtcatgaaggtttttcttttcctgagaaaacaacacgtattgttttctcaggttttgctttttggcctttttctagcttaaaaaaaaaaaaagcaaaattgtcttc

SEQ ID NO: 11 - DNA, 112 bp, synthetic construct
  misc_feature 1..112: note = Description of Artificial Sequence: Synthetic polynucleotide
  source 1..112: mol_type = other DNA
tcagtagggttgtaaaggtttttcttttcctgagaaaacaaccttttgttttctcaggttttgctttttggcctttccctagctttaaaaaaaaaaaagcaaaattgtcttc

SEQ ID NO: 12 - DNA, 68 bp, synthetic construct
  misc_feature 1..68: note = Description of Artificial Sequence: Synthetic oligonucleotide
  source 1..68: mol_type = other DNA
gaagtggcggttcggccggaggttccatcgtatccaaaaggctcttttcagagccacccattgtcttc

SEQ ID NO: 13 - DNA, 239 bp, synthetic construct
  misc_feature 1..239: note = Description of Artificial Sequence: Synthetic polynucleotide
  source 1..239: mol_type = other DNA
ggggctggcctcagtctctgtcccatcgcttgaatacagtactcctagggcttgaccctggtacccagcccagccttagcacccagcatgtgaccccactcctgatcaggtcccagcatcttcccttcttgttctgttccttaaggtcccagcaccttaccccaggacttggtcttcaaccaccattacccctctaactttgcacaaataaacctgtgtagaaacccaccccaaaaaaa

SEQ ID NO: 14 - DNA, 2100 bp, synthetic construct
  misc_feature 1..2100: note = Description of Artificial Sequence: Synthetic polynucleotide
  source 1..2100: mol_type = other DNA
atgatcccagcaagcgccaaggcaccacacaagcagccccacaagcagagcatctccatcggcaggggcacaaggaagagggacgaggatagcggaaccgaagtgggagagggaacagacgagtgggcacagtccaaggcaaccgtgcgcccacctgaccagctggagctgacagatgccgagctgaaggaggagttcaccaggatcctgacagccaacaatccacacgccccccagaacatcgtgcgctactctttcaaggagggcacatataagccaatcggctttgtgaaccagctggccgtgcactatacccaagtgggcaatctgatccccaaggactccgatgagggccggagacagcactacagggacgagctggtggcaggatcccaggagtctgtgaaagtgatctctgagaccggcaatctggaggaggacgaggagccaaaggagctggagaccgagccaggaagccagacagatgtgcctgcagcaggagcagcagagaaggtgaccgaggaggagctgatgacacctaagcagccaaaggagcggaagctgaccaaccagttcaatttttccgagagagcctctcagacatacaacaatccagtgcgggacagagagtgccagaccgagccaccccctagaaccaacttttccgccacagccaatcagtgggagatctacgatgcctatgtggaggagctggagaagcaggagaagaccaaggagaaggagaaggccaagacacccgtggccaagaagtccggcaagatggccatgcggaagctgaccagcatggagtcccagacagacgatctgatcaagctgtctcaggccgccaagatcatggagagaatggtgaaccagaatacctatgacgatatcgcccaggacttcaagtactatgacgatgcagcagacgagtacagggatcaagtgggcacactgctgcctctgtggaagtttcagaacgataaggccaagaggctgagcgtgaccgccctgtgctggaatccaaagtacagggacctgttcgcagtgggatacggatcttatgacttcatgaagcagagcagaggcatgctgctgctgtattccctgaagaacccctctttccctgagtacatgtttagctccaattccggcgtgatgtgcctggacatccacgtggatcacccctacctggtggccgtgggccactatgacggcaacgtggccatctacaatctgaagaagcctcactctcagcccagcttctgttctagcgccaagagcggcaagcactccgatcccgtgtggcaggtgaagtggcagaaggacgatatggaccagaacctgaatttcttttccgtgtcctctgatggcaggatcgtgtcttggaccctggtgaagcgcaagctggtgcacatcgacgtgatcaagctgaaggtggagggcagcaccacagaggtgccagagggactgcagctgcacccagtgggatgcggcacagccttcgactttcacaaggagatcgattatatgttcctggtgggcaccgaggagggcaagatctacaagtgttctaagagctatagctcccagtttctggacacatatgatgcccacaacatgagcgtggataccgtgtcctggaatccttaccacacaaaggtgttcatgagctgctctagcgactggaccgtgaagatctgggatcacaccatcaagacacctatgtttatctatgacctgaactccgccgtgggcgatgtggcatgggcaccatactcctctacagtgttcgcagcagtgaccacagacggcaaggcacacatctttgatctggccatcaacaagtacgaggccatctgtaatcagcccgtggccgccaagaagaacaggctgacccacgtgcagttcaatctgatccaccctatcatcatcgtgggcgacgatcggggccacatcatctctctgaagctgagccccaacctgagaaagatgcctaaggagaagaagggacaggaggtgcagaagggaccagcagtggagatcgcaaagctggacaagctgctgaatctggtgcgcgaggtgaagatcaagacctga

SEQ ID NO: 15 - DNA, 2100 bp, synthetic construct
  misc_feature 1..2100: note = Description of Artificial Sequence: Synthetic polynucleotide
  source 1..2100: mol_type = other DNA
atgatcccagcaagcgccaaggcaccacacaagcagccccacaagcagagcatcagcatcggcaggggcacaaggaagagggacgaggacagcggaaccgaagtgggagagggaacagacgagtgggcacagagcaaggcaaccgtgcgcccacccgaccagctggagctgacagacgccgagctgaaggaggagttcaccaggatcctgacagccaacaacccacacgccccccagaacatcgtgcgctacagcttcaaggagggcacatacaagccaatcggcttcgtgaaccagctggccgtgcactacacccaagtgggcaacctgatccccaaggacagcgacgagggccggagacagcactacagggacgagctggtggcaggaagccaggagagcgtgaaagtgatcagcgagaccggcaacctggaggaggacgaggagccaaaggagctggagaccgagccaggaagccagacagacgtgcccgcagcaggagcagcagagaaggtgaccgaggaggagctgatgacacccaagcagccaaaggagcggaagctgaccaaccagttcaacttcagcgagagagccagccagacatacaacaacccagtgcgggacagagagtgccagaccgagccaccccccagaaccaacttcagcgccacagccaaccagtgggagatctacgacgcctacgtggaggagctggagaagcaggagaagaccaaggagaaggagaaggccaagacacccgtggccaagaagagcggcaagatggccatgcggaagctgaccagcatggagagccagacagacgacctgatcaagctgagccaggccgccaagatcatggagagaatggtgaaccagaacacctacgacgacatcgcccaggacttcaagtactacgacgacgcagcagacgagtacagggaccaagtgggcacactgctgcccctgtggaagttccagaacgacaaggccaagaggctgagcgtgaccgccctgtgctggaacccaaagtacagggacctgttcgcagtgggatacggaagctacgacttcatgaagcagagcagaggcatgctgctgctgtacagcctgaagaaccccagcttccccgagtacatgttcagcagcaacagcggcgtgatgtgcctggacatccacgtggaccacccctacctggtggccgtgggccactacgacggcaacgtggccatctacaacctgaagaagccccacagccagcccagcttctgcagcagcgccaagagcggcaagcacagcgaccccgtgtggcaggtgaagtggcagaaggacgacatggaccagaacctgaacttcttcagcgtgagcagcgacggcaggatcgtgagctggaccctggtgaagcgcaagctggtgcacatcgacgtgatcaagctgaaggtggagggcagcaccacagaggtgccagagggactgcagctgcacccagtgggatgcggcacagccttcgacttccacaaggagatcgactacatgttcctggtgggcaccgaggagggcaagatctacaagtgcagcaagagctacagcagccagttcctggacacatacgacgcccacaacatgagcgtggacaccgtgagctggaacccctaccacacaaaggtgttcatgagctgcagcagcgactggaccgtgaagatctgggaccacaccatcaagacacccatgttcatctacgacctgaacagcgccgtgggcgacgtggcatgggcaccatacagcagcacagtgttcgcagcagtgaccacagacggcaaggcacacatcttcgacctggccatcaacaagtacgaggccatctgcaaccagcccgtggccgccaagaagaacaggctgacccacgtgcagttcaacctgatccaccccatcatcatcgtgggcgacgaccggggccacatcatcagcctgaagctgagccccaacctgagaaagatgcccaaggagaagaagggacaggaggtgcagaagggaccagcagtggagatcgcaaagctggacaagctgctgaacctggtgcgcgaggtgaagatcaagacctga

SEQ ID NO: 16 - DNA, 2100 bp, synthetic construct
  misc_feature 1..2100: note = Description of Artificial Sequence: Synthetic polynucleotide
  source 1..2100: mol_type = other DNA
atgatcccagcaagcgccaaggcaccacacaagcagccccacaagcagagcatctccatcggcaggggcacaaggaagagggacgaggacagcggaaccgaagtgggagagggaacagacgagtgggcacagtccaaggcaaccgtgcgcccacctgaccagctggagctgacagatgccgagctgaaggaggagttcaccaggatcctgacagccaacaatccacacgccccccagaacatcgtgcgctacagcttcaaggagggcacatacaagccaatcggcttcgtgaaccagctggccgtgcactacacccaagtgggcaatctgatccccaaggactccgatgagggccggagacagcactacagggacgagctggtggcaggatcccaggagtctgtgaaagtgatctctgagaccggcaatctggaggaggacgaggagccaaaggagctggagaccgagccaggaagccagacagatgtgcctgcagcaggagcagcagagaaggtgaccgaggaggagctgatgacacccaagcagccaaaggagcggaagctgaccaaccagttcaacttctccgagagagcctctcagacatacaacaatccagtgcgggacagagagtgccagaccgagccaccccccagaaccaacttctccgccacagccaatcagtgggagatctacgatgcctacgtggaggagctggagaagcaggagaagaccaaggagaaggagaaggccaagacacccgtggccaagaagtccggcaagatggccatgcggaagctgaccagcatggagtcccagacagacgatctgatcaagctgtctcaggccgccaagatcatggagagaatggtgaaccagaacacctacgacgacatcgcccaggacttcaagtactacgacgatgcagcagacgagtacagggatcaagtgggcacactgctgcctctgtggaagttccagaacgacaaggccaagaggctgagcgtgaccgccctgtgctggaatccaaagtacagggacctgttcgcagtgggatacggaagctacgacttcatgaagcagagcagaggcatgctgctgctgtactccctgaagaaccccagcttccctgagtacatgttcagctccaactccggcgtgatgtgcctggacatccacgtggatcacccctacctggtggccgtgggccactacgacggcaacgtggccatctacaatctgaagaagcctcactctcagcccagcttctgcagcagcgccaagagcggcaagcactccgatcccgtgtggcaggtgaagtggcagaaggacgacatggaccagaacctgaacttcttctccgtgtcctctgatggcaggatcgtgagctggaccctggtgaagcgcaagctggtgcacatcgacgtgatcaagctgaaggtggagggcagcaccacagaggtgccagagggactgcagctgcacccagtgggatgcggcacagccttcgacttccacaaggagatcgactacatgttcctggtgggcaccgaggagggcaagatctacaagtgcagcaagagctacagctcccagttcctggacacatacgatgcccacaacatgagcgtggacaccgtgtcctggaatccctaccacacaaaggtgttcatgagctgcagcagcgactggaccgtgaagatctgggatcacaccatcaagacacccatgttcatctacgacctgaactccgccgtgggcgatgtggcatgggcaccatactccagcacagtgttcgcagcagtgaccacagacggcaaggcacacatcttcgatctggccatcaacaagtacgaggccatctgcaatcagcccgtggccgccaagaagaacaggctgacccacgtgcagttcaatctgatccaccccatcatcatcgtgggcgacgatcggggccacatcatctctctgaagctgagccccaacctgagaaagatgcccaaggagaagaagggacaggaggtgcagaagggaccagcagtggagatcgcaaagctggacaagctgctgaatctggtgcgcgaggtgaagatcaagacctga

SEQ ID NO: 17 - DNA, 13875 bp, synthetic construct
  misc_feature 1..13875: note = Description of Artificial Sequence: Synthetic polynucleotide
  source 1..13875: mol_type = other DNA
atgttcagaatcggcagacggcagctgtggaagcacagcgtgaccagagtgctgacccagcggctgaagggcgagaaagaggccaagagagccctgctggacgcccggcacaactacctgttcgccatcgtggccagctgcctggacctgaacaagaccgaggtggaagacgccatcctggaaggcaaccagatcgagcggatcgaccagctgttcgccgtgggcggactgcggcacctgatgttctactaccaagacgtggaagaggccgagacaggccagctgggaagcctgggcggagtgaacctggtgagcggcaagatcaagaaacccaaggtgttcgtgaccgagggcaacgacgtggccctgacaggcgtgtgcgtgttcttcatcagaaccgaccccagcaaggccatcacccccgacaacatccaccaggaagtgagcttcaacatgctggacgccgccgacggcggcctgctgaacagcgtgcggagactgctgagcgacatcttcatccccgccctgagagccacaagccacggctggggagagctggaaggactgcaggacgccgccaacatccggcaggaattcctgagcagcctggaaggattcgtgaacgtgctgagcggcgcccaggaaagcctgaaagaaaaagtgaacctgcggaagtgcgacatcctggaactgaaaaccctgaaagagcccaccgactacctgaccctggccaacaaccccgagacactgggcaagatcgaggactgcatgaaagtgtggatcaagcagaccgaacaggtgctggccgagaacaaccagctgctgaaagaagccgacgacgtgggcccaagagccgagctggaacactggaagaagcggctgagcaagttcaactacctgctggaacagctgaagagccccgacgtgaaggccgtgctggccgtgctggcagccgccaagagcaaactgctgaaaacctggcgcgagatggacatccggatcaccgacgccaccaacgaggccaaggacaacgtgaagtacctgtacaccctggaaaagtgctgcgaccccctgtacagcagcgaccccctgagcatgatggacgccatccccaccctgatcaacgccatcaagatgatctacagcatcagccactactacaacaccagcgagaagatcaccagcctgttcgtgaaagtgaccaaccagatcatcagcgcctgcaaggcctacatcaccaacaacggcaccgccagcatctggaaccagccccaggacgtggtggaagagaagatcctgagcgccatcaagctgaagcaggaataccagctgtgcttccacaagaccaagcagaagctgaaacagaaccccaacgccaagcagttcgacttcagcgagatgtacatcttcggcaagttcgagacattccaccggcggctggccaagatcatcgacatcttcaccaccctgaaaacatacagcgtgctgcaggacagcaccatcgagggcctggaagacatggccaccaagtaccagggcatcgtggccaccatcaagaagaaagagtacaacttcctggaccagcgcaagatggacttcgaccaggactacgaggaattctgcaagcagacaaacgacctgcacaacgagctgcgcaagttcatggacgtgaccttcgccaagatccagaacaccaaccaggccctgcggatgctgaagaagttcgagagactgaacatccccaacctgggcatcgacgacaagtaccagctgatcctggaaaactacggcgccgacatcgacatgatcagcaagctgtacacaaagcagaagtacgacccccccctggcccggaaccagccccccatcgccggcaaaatcctgtgggccagacagctgttccaccggatccagcagcccatgcagctgttccagcagcaccccgccgtgctgagcacagccgaggccaaacccatcatccggagctacaaccggatggccaaggtgctgctggaattcgaggtgctgttccaccgggcctggctgcggcagatcgaagagatccacgtgggactggaagccagcctgctcgtgaaggcccccggaaccggcgagctgttcgtgaacttcgacccccagatcctgatcctgttccgggaaaccgagtgcatggcccagatggggctggaagtgagccccctggccaccagcctgttccagaagcgggaccggtacaagcggaacttcagcaacatgaagatgatgctggccgagtaccagcgcgtgaagagcaagatccccgccgccatcgagcagctgatcgtgccccacctggccaaagtggacgaggccctgcagccaggactggccgccctgacatggaccagcctgaacatcgaggcctacctggaaaacacattcgccaaaatcaaggacctggaactgctgctggaccgcgtgaacgacctgatcgagttccggatcgacgccatcctggaagagatgagcagcacccccctgtgccagctgccccaggaagaacccctgacctgcgaagagttcctgcagatgaccaaggacctgtgcgtgaacggcgcccagatcctgcacttcaagagcagcctggtggaagaagccgtgaacgagctcgtgaacatgctgctggacgtggaagtgctgagcgaggaagagagcgagaagatcagcaacgagaacagcgtgaactacaagaacgagagcagcgccaagcgggaagagggcaacttcgacaccctgaccagcagcatcaacgccagagccaacgccctgctgctgaccaccgtgacccggaagaaaaaagaaaccgagatgctgggcgaagaggccagagagctgctgagccacttcaaccaccagaacatggacgccctgctgaaagtgacacggaacaccctggaagccatccggaagcggatccacagcagccacaccatcaacttccgggacagcaacagcgccagcaacatgaagcagaacagcctgcccatcttccgggccagcgtgacactggccatccccaacatcgtgatggcccccgccctggaagacgtgcagcagacactgaacaaggccgtggaatgcatcatcagcgtgcccaagggcgtgcggcagtggagcagcgaactgctgagcaagaagaagatccaggaacggaaaatggccgccctgcagagcaacgaggacagcgacagcgacgtggaaatgggcgagaacgagctgcaggacacactggaaatcgccagcgtgaacctgcccatccccgtgcagaccaagaactactacaagaacgtgagcgaaaacaaagaaatcgtgaagctggtgagcgtgctgagcaccatcatcaacagcaccaagaaagaagtgatcaccagcatggactgcttcaagcggtacaaccacatctggcagaagggcaaagaagaggccatcaagaccttcatcacccagagccccctgctgagcgagttcgagagccagatcctgtacttccagaacctggaacaggaaatcaacgccgagcccgagtacgtgtgcgtgggcagcatcgccctgtacaccgccgacctgaagttcgccctgaccgccgagacaaaggcctggatggtcgtgatcggccggcactgcaacaaaaagtacagaagcgagatggaaaacatcttcatgctgatcgaggaattcaacaagaaactgaaccggcccatcaaggacctggacgacatcagaatcgccatggccgcactgaaagagatcagagaggaacagatcagcatcgacttccaagtgggccccatcgaggaaagctacgccctgctgaacagatacggactgctgatcgcccgggaagagatcgacaaggtggacaccctgcactacgcctgggagaagctgctggccagagccggcgaggtgcagaacaaactggtgagcctgcagcccagcttcaagaaagaactgatcagcgccgtggaagtgttcctgcaggactgccaccagttctacctggactacgacctgaacggccccatggccagcggcctgaaaccccaggaagccagcgaccggctgatcatgttccagaaccagttcgacaacatctaccggaagtacatcacctacacaggcggcgaggaactgttcggcctgcccgccacacagtacccccagctgctggaaatcaagaagcagctgaacctgctgcagaagatctacaccctgtacaacagcgtgatcgagacagtgaacagctactacgacatcctgtggagcgaagtgaacatcgagaagatcaacaacgaactgctggaattccagaaccggtgccggaagctgcccagagcactgaaggactggcaggccttcctggacctgaagaaaatcatcgacgacttcagcgagtgctgccccctgctggagtacatggccagcaaggccatgatggaacggcactgggagagaatcaccacactgaccggccacagcctggacgtgggcaacgagagcttcaagctgcggaacatcatggaagccccactgctgaagtacaaagaggaaatcgaggacatctgcatcagcgccgtgaaagagcgggacatcgagcagaaactgaaacaagtgatcaacgagtgggacaacaagaccttcaccttcggcagcttcaagaccagaggcgagctgctgctgcggggcgacagcaccagcgagatcatcgccaacatggaagacagcctgatgctgctgggcagcctgctgagcaaccggtacaacatgcccttcaaggcccagatccagaaatgggtgcagtacctgagcaacagcaccgacatcatcgagagctggatgaccgtgcagaacctgtggatctacctggaagccgtgttcgtgggcggcgacatcgccaagcagctgcccaaagaggccaagcggttcagcaacatcgacaagagctgggtcaagatcatgaccagagcccacgaggtgcccagcgtggtgcagtgctgcgtgggcgacgaaacactgggacagctgctgccccacctgctggaccagctggaaatctgccagaagagcctgaccggctacctggaaaagaaacggctgtgcttcccccggttcttcttcgtgagcgaccccgccctgctggaaatcctgggccaggccagcgacagccacacaatccaggcccacctgctgaacgtgttcgacaacatcaagagcgtgaagttccacgagaaaatctacgaccggatcctgagcatcagcagccaggaaggcgagacaatcgagctggacaagcccgtgatggccgagggaaacgtggaagtgtggctgaacagcctgctggaagagagccagagcagcctgcacctcgtgatcagacaggccgccgccaacatccaggaaaccggcttccagctgaccgagttcctgagcagcttcccagcacaagtgggactgctgggcatccagatgatctggaccagagacagcgaagaggccctgagaaacgccaagttcgacaagaaaatcatgcagaaaacaaaccaggcattcctggaactgctgaacaccctgatcgacgtgaccacccgggacctgagcagcaccgagagagtgaagtacgagacactgatcaccatccacgtgcaccagcgggacatcttcgacgacctgtgccacatgcacatcaagagccccatggacttcgagtggctgaagcagtgcaggttctacttcaacgaggacagcgacaagatgatgatccacatcaccgacgtggccttcatctaccagaacgagttcctgggctgcaccgaccgcctcgtgatcacccccctgaccgaccggtgctacatcacactggcccaggcactgggcatgagcatgggaggcgcaccagcaggacccgccggcacaggcaagaccgaaaccaccaaggacatgggacgctgcctgggcaaatacgtggtggtgttcaactgcagcgaccagatggacttccggggcctgggccggatcttcaagggcctggcacagagcggaagctggggctgcttcgacgagttcaacagaatcgacctgcccgtgctgagcgtggccgcacagcagatcagcatcatcctgacatgcaaaaaagagcacaagaagagcttcatcttcaccgacggcgacaacgtgaccatgaaccccgagttcggcctgttcctgacaatgaaccccggctacgccggacggcaggaactgcccgagaacctgaagatcaacttccggagcgtggccatgatggtgcccgaccggcagatcatcatcagagtgaaactggccagctgcggcttcatcgacaacgtggtgctggcccggaagttcttcacactgtacaagctgtgcgaagaacagctgagcaaacaggtgcactacgacttcggcctgaggaacatcctgagcgtgctgagaaccctgggagccgccaagcgggccaaccccatggacaccgagagcacaatcgtgatgcgggtgctgcgggacatgaacctgagcaagctgatcgacgaggacgagcccctgttcctgagcctgatcgaggacctgttccccaacatcctgctggacaaggccggctaccccgaactggaagccgccatcagcagacaggtggaagaggccggcctgatcaaccaccccccctggaaactgaaagtgatccagctgttcgagacacagcgcgtgcggcacggcatgatgacactgggacccagcggagccggcaagaccacctgcatccacacactgatgcgggccatgaccgactgcggcaagccccaccgcgagatgcggatgaaccccaaggccatcaccgccccccagatgttcggcagactggacgtggccaccaacgactggaccgacggcatcttcagcaccctgtggcgcaagaccctgcgggccaagaagggcgagcacatctggatcatcctggacggccccgtggacgccatctggatcgagaacctgaacagcgtgctggacgacaacaagacactgaccctggccaacggcgaccggatccccatggcccccaactgcaagatcatcttcgagccccacaacatcgacaacgccagccccgccaccgtgagcagaaacggcatggtgttcatgagcagcagcatcctggactggagccccatcctggaaggcttcctgaagaagcggagcccccaggaagccgagatcctgagacagctgtacaccgagagcttccccgacctgtaccggttctgcatccagaacctggagtacaagatggaagtgctggaagccttcgtgatcacccagagcatcaacatgctgcagggcctgatccccctgaaagaacagggcggagaagtgagccaggcccacctgggcagactgttcgtgttcgccctgctgtggagcgccggcgccgccctggaactggacggaaggcggagactggaactgtggctgcggagcagacccaccggcaccctggaactgcccccaccagccggacccggcgacaccgccttcgactactacgtggcccccgacggcacctggacccactggaacacccggacccaggaatacctgtaccccagcgacaccacccccgagtacggcagcatcctggtgcccaacgtggacaacgtgcggaccgacttcctgatccagacaatcgccaagcagggaaaggccgtgctgctgatcggcgagcagggcacagccaagaccgtgatcatcaagggcttcatgagcaagtacgaccccgagtgccacatgatcaagagcctgaacttcagcagcgccaccaccccactgatgttccagcggaccatcgagagctacgtggacaagcggatgggcaccacctacggccccccagccggcaagaaaatgaccgtgttcatcgacgacgtgaacatgcccatcatcaacgagtggggcgaccaagtgaccaacgagatcgtgcggcagctgatggaacagaacggcttctacaacctggaaaagcccggcgagttcaccagcatcgtggacatccagttcctggccgccatgatccaccccggcggcggaagaaacgacatcccccagcggctgaagcggcagttcagcatcttcaactgcaccctgcccagcgaggccagcgtggacaagatcttcggcgtgatcggcgtgggccactactgcacccagagaggcttcagcgaggaagtgcgggacagcgtgaccaagctggtgcccctgacaagacggctgtggcagatgaccaagatcaagatgctgcccacccccgccaagttccactacgtgttcaacctgcgggacctgagcagagtgtggcagggaatgctgaacaccaccagcgaagtgatcaaagagcccaacgacctgctgaagctgtggaagcacgagtgcaagagagtgatcgccgaccggttcaccgtgagcagcgacgtgacatggttcgacaaggccctggtgagcctggtggaagaggaattcggcgaagagaagaaactgctggtggactgcggcatcgacacctacttcgtggacttcctgcgcgacgcccccgaagccgccggcgagacaagcgaagaggccgacgccgagacacccaagatctacgagcccatcgagagcttcagccacctgaaagaaaggctgaacatgttcctgcagctgtacaacgagagcatccggggagccggcatggacatggtgttcttcgccgacgccatggtgcacctcgtgaagatcagcagagtgatccggaccccccagggcaacgccctgctcgtgggagtgggaggcagcggcaagcagagcctgaccagactggccagcttcatcgccggctacgtgagcttccagatcaccctgacccggagctacaacaccagcaacctgatggaagacctgaaggtgctgtaccggacagccggccagcaggggaagggcatcaccttcatcttcaccgacaacgagatcaaggacgagagcttcctggagtacatgaacaacgtgctgagcagcggcgaggtgagcaacctgttcgcccgggacgagatcgacgagatcaacagcgacctggccagcgtgatgaagaaagaattcccccggtgcctgcccacaaacgagaacctgcacgactacttcatgagcagagtgcggcagaacctgcacatcgtgctgtgcttcagccccgtgggcgagaagttcagaaaccgggccctgaagttccccgccctgatcagcggctgcaccatcgactggttcagccggtggcccaaggacgccctggtggccgtgagcgagcacttcctgaccagctacgacatcgactgcagcctggaaatcaagaaagaggtggtgcagtgcatgggcagcttccaggacggcgtggccgagaaatgcgtggactacttccagcggttccggcggagcacccacgtgacccccaagagctacctgagcttcatccagggctacaagttcatctacggcgagaagcacgtggaagtgcgcacactggccaaccggatgaacaccggcctggaaaaactgaaagaggccagcgagagcgtggccgccctgagcaaagaactggaagccaaagaaaaagaactgcaggtggccaacgacaaggccgacatggtgctgaaagaagtgaccatgaaggcccaggccgccgagaaagtgaaagccgaggtgcagaaagtgaaggaccgggcccaggccatcgtggacagcatcagcaaggacaaggccatcgccgaggaaaagctggaagcagccaagcccgccctggaagaggcagaagccgccctgcagaccatccggcccagcgacatcgccacagtgcggaccctgggaaggcccccccacctgatcatgcggatcatggactgcgtgctgctgctgttccagagaaaggtgagcgccgtgaagatcgacctggaaaaaagctgcaccatgcccagctggcaggaaagcctgaagctgatgaccgccggcaacttcctgcagaacctgcagcagttccccaaggacaccatcaacgaggaagtgatcgagttcctgagcccctacttcgagatgcccgactacaacatcgaaaccgccaaacgcgtgtgcggcaacgtggccggactgtgcagctggaccaaggccatggccagcttcttcagcatcaacaaagaggtgctgcccctgaaggccaacctggtggtgcaggaaaaccggcacctgctggccatgcaggacctgcagaaagcccaggccgagctggacgacaagcaggccgagctggacgtggtgcaggccgagtacgagcaggccatgaccgagaagcagaccctgctggaagacgcagagcggtgcagacacaagatgcagaccgccagcaccctgatcagcggactggccggcgaaaaagagcggtggaccgagcagagccaggaattcgccgcccagaccaagcggctcgtgggagacgtgctgctggccaccgccttcctgagctacagcggccccttcaaccaggaattcagggacctgctgctgaacgactggcggaaagagatgaaggccagaaagatccccttcggcaagaacctgaacctgagcgagatgctgatcgacgcccccaccatcagcgagtggaacctgcagggactgcccaacgacgacctgagcatccagaacggaatcatcgtgaccaaagccagcagataccccctgctgatcgacccccagacacagggcaagatctggatcaagaacaaagagagccggaacgagctgcagatcaccagcctgaaccacaagtacttccggaaccacctggaagacagcctgagcctgggcaggccactgctgatcgaggacgtgggcgaggaactggacccagccctggacaacgtgctggaacggaacttcatcaagaccggcagcaccttcaaagtgaaagtgggcgacaaagaagtggacgtgctggacggcttccggctgtacatcaccaccaagctgcccaaccccgcctacacccccgagatcagcgcccggaccagcatcatcgacttcaccgtgacaatgaagggactggaagaccagctgctgggacgcgtgatcctgacagagaagcaggaactggaaaaagaacggacccacctgatggaagacgtgaccgccaacaagcggcggatgaaggaactggaagacaacctgctgtacaggctgaccagcacccagggcagcctggtggaagacgagagcctgatcgtggtgctgagcaacaccaagcggaccgcagaggaagtgacccagaagctggaaatcagcgccgagacagaggtgcagatcaacagcgccagagaagagtaccggcccgtggccacccggggaagcatcctgtacttcctgatcaccgagatgcggctcgtgaacgagatgtaccagaccagcctgcggcagttcctgggcctgttcgacctgagcctggccagaagcgtgaagagccccatcaccagcaagagaatcgccaacatcatcgagcacatgacctacgaggtgtacaaatacgccgccagaggcctgtacgaggaacacaagttcctgttcacactgctgctgaccctgaagatcgacatccagcggaacagagtgaagcacgaagagttcctgacactgatcaaggggggagccagcctggacctgaaggcctgcccccccaagcccagcaagtggatcctggacatcacctggctgaacctggtggaactgagcaagctgagacagttcagcgacgtgctggaccagatcagccgcaacgagaagatgtggaagatctggttcgacaaagagaaccccgaggaagaacccctgcccaacgcctacgacaagagcctggactgcttccggcggctgctgctgatcagaagctggtgccccgaccggacaatcgcccaggcccgcaagtacatcgtggacagcatgggagagaagtacgccgagggcgtgatcctggacctggaaaagacctgggaggaaagcgaccccagaacccccctgatctgcctgctgagcatgggcagcgaccccaccgacagcatcatcgccctgggcaagagactgaagatcgagacaagatacgtgagcatgggccagggccaggaagtgcacgccagaaagctgctgcagcagaccatggccaacggcggctgggccctgctgcagaactgccacctggggctggacttcatggacgaactgatggacatcatcatcgagacagagctggtgcacgacgccttcagactgtggatgaccaccgaggcccacaagcagttccccatcaccctgctgcagatgagcatcaagttcgccaacgaccccccccagggactgagagccggcctgaagagaacctacagcggcgtgagccaggacctgctggacgtgagcagcggcagccagtggaagcccatgctgtacgccgtggcattcctgcacagcaccgtgcaggaacggcggaagttcggcgccctgggatggaacatcccctacgagttcaaccaggccgacttcaacgccaccgtgcagttcatccagaaccacctggacgacatggacgtgaagaaaggggtgagctggacaaccatccggtacatgatcggagagatccagtacggcggcagagtgaccgacgactacgacaagaggctgctgaacaccttcgccaaagtgtggttcagcgagaacatgttcggccccgacttcagcttctaccagggctacaacatccccaagtgcagcaccgtggacaactacctgcagtacatccagagcctgcccgcctacgacagccccgaggtgttcggactgcaccccaacgccgacatcacctaccagagcaaactggccaaggacgtgctggacaccatcctgggcatccagcccaaggacaccagcggcggaggcgacgaaacccgggaagcagtggtggccagactggccgacgacatgctggaaaagctgccccccgactacgtgcccttcgaagtgaaagaacgcctgcagaagatgggccccttccagcccatgaacatcttcctgaggcaggaaatcgaccggatgcagcgggtgctgagcctcgtgcggagcacactgaccgagctgaaactggccatcgacggcaccatcatcatgagcgagaacctgcgggacgcactggactgcatgttcgacgccagaatccccgcatggtggaaaaaggccagctggatcagcagcaccctgggcttctggttcaccgaactgatcgagagaaacagccagttcaccagctgggtgttcaacggcagaccccactgcttctggatgaccggcttcttcaacccacaaggcttcctgacagcaatgcgccaggaaatcaccagagccaacaagggctgggccctggacaacatggtgctgtgcaacgaagtgaccaagtggatgaaggacgacatcagcgccccccccacagagggcgtgtacgtgtacggcctgtacctggaaggcgccggatgggacaagagaaacatgaagctgatcgagagcaagcccaaggtgctgttcgagctgatgcccgtgatcaggatctacgccgagaacaacaccctgagggacccccggttctacagctgccccatctacaagaaacccgtgcgcaccgacctgaactacatcgccgccgtggacctgaggacagcccagacacccgagcactgggtgctgagaggcgtggcactgctgtgcgacgtgaagtga

SEQ ID NO: 18 - DNA, 13875 bp, synthetic construct
  misc_feature 1..13875: note = Description of Artificial Sequence: Synthetic polynucleotide
  source 1..13875: mol_type = other DNA
atgttcagaatcggcagacggcagctgtggaagcacagcgtgaccagagtgctgacccagcggctgaagggcgagaaagaggccaagagagccctgctggacgcccggcacaattacctgtttgccatcgtggccagctgcctggacctgaacaagaccgaggtggaagatgccatcctggaaggcaaccagatcgagcggatcgaccagctgtttgccgtgggcggactgcggcacctgatgttctattatcaagacgtggaagaggccgagacaggccagctgggatctctgggcggagtgaatctggtgtccggcaagatcaagaaacccaaggtgttcgtgaccgagggcaacgacgtggccctgacaggcgtgtgcgtgttcttcatcagaaccgaccccagcaaggccatcacccccgacaacatccaccaggaagtgtccttcaacatgctggatgccgccgatggcggcctgctgaattctgtgcggagactgctgagcgacatcttcatccccgccctgagagccacatctcacggctggggagagctggaaggactgcaggacgccgccaatatccggcaggaatttctgagcagcctggaaggattcgtgaacgtgctgtctggcgcccaggaaagcctgaaagaaaaagtgaacctgcggaagtgcgatatcctggaactgaaaaccctgaaagagcccaccgactacctgaccctggccaacaaccctgagacactgggcaagatcgaggactgcatgaaagtgtggatcaagcagaccgaacaggtgctggccgagaacaaccagctgctgaaagaagccgacgacgtgggcccaagagccgagctggaacactggaagaagcggctgagcaagttcaactacctgctggaacagctgaagtcccccgacgtgaaggccgtgctggctgtgctggcagccgccaagagcaaactgctgaaaacctggcgcgagatggacatccggatcaccgacgccaccaacgaggccaaggacaacgtgaagtacctgtacaccctggaaaagtgctgcgaccccctgtacagcagcgaccctctgagcatgatggacgccatccctaccctgatcaacgccatcaagatgatctacagcatcagccactactacaacaccagcgagaagatcaccagcctgttcgtgaaagtgaccaatcagatcatcagcgcctgcaaggcctacatcaccaacaacggcaccgccagcatctggaaccagccccaggatgtggtggaagagaagatcctgtctgccatcaagctgaagcaggaataccagctgtgttttcacaagaccaagcagaagctgaaacagaaccccaacgccaagcagttcgacttcagcgagatgtatatcttcggcaagttcgagacattccaccggcggctggccaagatcatcgacatctttaccaccctgaaaacatacagcgtgctgcaggacagcaccatcgagggcctggaagatatggccaccaagtaccagggcattgtggccaccatcaagaagaaagagtacaacttcctggaccagcgcaagatggacttcgaccaggactacgaggaattctgcaagcagacaaacgacctgcacaacgagctgcgcaagtttatggacgtgaccttcgccaagatccagaacaccaaccaggccctgcggatgctgaagaagtttgagagactgaacatccccaacctgggcatcgacgataagtaccagctgatcctggaaaactacggcgccgacatcgacatgatcagcaagctgtacacaaagcagaagtacgacccccccctggcccggaatcagcctcctatcgccggcaaaatcctgtgggctagacagctgtttcaccggatccagcagcccatgcagctgttccagcagcaccctgccgtgctgagcacagccgaggccaaacccatcatccggtcctacaaccggatggccaaggtgctgctggaattcgaggtgctgttccaccgggcctggctgcggcagatcgaagagattcacgtgggactggaagccagcctgctcgtgaaggctcctggaaccggcgagctgtttgtgaacttcgacccccagatcctgatcctgttccgggaaaccgagtgcatggcccagatggggctggaagtgtctcctctggccacctccctgttccagaagcgggaccggtacaagcggaacttcagcaacatgaagatgatgctggctgagtaccagcgcgtgaagtccaagatccccgctgccatcgagcagctgatcgtgcctcacctggccaaagtggacgaggccctgcagccaggactggccgctctgacatggaccagcctgaacatcgaggcctatctggaaaacacattcgccaaaatcaaggatctggaactgctgctggaccgcgtgaacgacctgatcgagttccggatcgacgccattctggaagagatgtccagcacccccctgtgtcagctgccccaggaagaacccctgacctgcgaagagttcctgcagatgaccaaggacctgtgcgtgaacggcgcccagattctgcacttcaagtccagcctggtggaagaagccgtgaacgagctcgtgaatatgctgctggatgtggaagtgctgagcgaggaagagtccgagaagatctccaacgagaacagcgtgaactacaagaacgagtccagcgccaagcgggaagagggcaacttcgacaccctgaccagctccatcaatgccagagccaacgccctgctgctgaccaccgtgacccggaagaaaaaagaaaccgagatgctgggcgaagaggctagagagctgctgtcccacttcaaccaccagaacatggatgccctgctgaaagtgacacggaataccctggaagccatccggaagcggatccacagcagccacaccatcaacttccgggacagcaacagcgccagcaatatgaagcagaacagcctgcccatcttccgggcctccgtgacactggccatccccaatatcgtgatggcccctgctctggaagatgtgcagcagacactgaacaaggccgtggaatgcatcatctccgtgcccaagggcgtgcggcagtggtctagcgaactgctgtccaagaagaagatccaggaacggaaaatggccgccctgcagtctaacgaggacagcgactccgacgtggaaatgggcgagaatgagctgcaggatacactggaaatcgcctctgtgaatctgcccatccccgtgcagaccaagaactactataagaacgtgtccgaaaacaaagaaatcgtgaagctggtgtctgtgctgtccaccatcatcaacagcaccaagaaagaagtgatcacctccatggactgcttcaagcggtacaaccacatctggcagaagggcaaagaagaggccattaagaccttcatcacccagagccccctgctgtccgagttcgagtctcagatcctgtacttccagaacctggaacaggaaatcaacgccgagcccgagtacgtgtgtgtgggctctatcgccctgtataccgccgacctgaagttcgccctgaccgccgagacaaaggcctggatggtcgtgatcggccggcactgcaacaaaaagtacagatccgagatggaaaacatctttatgctgattgaggaattcaacaagaaactgaaccggcccattaaggacctggacgacatcagaatcgccatggccgcactgaaagagatcagagaggaacagatcagcatcgacttccaagtgggccccatcgaggaaagctacgctctgctgaacagatacggactgctgatcgcccgggaagagatcgacaaggtggacaccctgcactacgcctgggagaagctgctggctagagccggcgaggtgcagaacaaactggtgtctctgcagcccagctttaagaaagaactgatctccgccgtggaagtgtttctgcaggactgccaccagttctacctggactacgacctgaacggccccatggcctctggcctgaaacctcaggaagcctccgaccggctgattatgtttcagaaccagttcgacaatatctaccggaagtacatcacctacacaggcggcgaggaactgttcggcctgcctgccacacagtacccccagctgctggaaatcaagaagcagctgaacctgctgcagaagatctacaccctgtacaactccgtgatcgagacagtgaacagctactacgacatcctgtggagcgaagtgaacattgagaagattaacaatgaactgctggaatttcagaaccggtgccggaagctgcccagagcactgaaggattggcaggcctttctggatctgaagaaaatcatcgacgacttctccgagtgctgccctctgctggagtacatggcctccaaggccatgatggaacggcactgggagagaatcaccacactgaccggccacagcctggacgtgggcaacgagagcttcaagctgcggaacatcatggaagccccactgctgaagtacaaagaggaaatcgaggacatctgtatcagcgccgtgaaagagcgggatatcgagcagaaactgaaacaagtgatcaacgagtgggacaacaagacctttaccttcggcagcttcaagaccagaggcgagctgctgctgcggggcgatagcacctctgagatcattgccaacatggaagatagcctgatgctgctgggctccctgctgagcaaccggtataacatgcccttcaaggctcagattcagaaatgggtgcagtacctgagcaactccaccgacatcatcgagtcctggatgaccgtgcagaacctgtggatctacctggaagccgtgttcgtgggcggcgacattgccaagcagctgcccaaagaggctaagcggttctccaacatcgacaagagctgggtcaagatcatgaccagagcccacgaggtgcccagcgtggtgcagtgctgtgtgggcgacgaaacactgggacagctgctgcctcatctgctggaccagctggaaatctgccagaagtccctgaccggctacctggaaaagaaacggctgtgtttcccccggttcttcttcgtgtccgaccccgccctgctggaaattctgggccaggccagcgactcacacacaattcaggcccatctgctgaatgtgttcgataacatcaagagcgtgaagttccacgagaaaatctacgaccggatcctgagcatcagctcccaggaaggcgagacaatcgagctggacaagcctgtgatggccgagggaaacgtggaagtgtggctgaacagcctgctggaagagtcccagagcagcctgcacctcgtgatcagacaggccgctgccaacatccaggaaaccggctttcagctgaccgagttcctgtccagcttcccagcacaagtgggactgctgggcatccagatgatttggaccagagactccgaagaggccctgagaaacgccaagttcgataagaaaattatgcagaaaacaaatcaggcatttctggaactgctgaacaccctgatcgacgtgaccacccgggacctgagcagcaccgagagagtgaagtacgagacactgatcaccatccacgtgcaccagcgggacatcttcgacgacctgtgccacatgcacatcaagtctcccatggatttcgagtggctgaagcagtgcaggttctacttcaacgaggactccgacaagatgatgatccacatcaccgatgtggcctttatctatcagaatgagttcctgggctgtaccgatcgcctcgtgattacccccctgaccgaccggtgttacatcacactggcccaggcactgggcatgtctatgggaggcgcaccagcaggacctgccggcacaggcaagaccgaaaccaccaaggacatgggacgctgcctgggcaaatacgtggtggtgttcaactgcagcgaccagatggatttccggggcctgggccggatctttaagggcctggcacagagcggaagctggggctgcttcgacgagttcaacagaatcgacctgcccgtgctgtccgtggccgcacagcagatctccatcatcctgacatgcaaaaaagagcacaagaagtccttcatcttcaccgacggcgacaatgtgaccatgaaccccgagtttggcctgttcctgacaatgaaccctggctacgccggacggcaggaactgcccgagaacctgaagatcaactttcggagtgtggctatgatggtgcccgaccggcagatcattatcagagtgaaactggcctcctgcggcttcatcgacaacgtggtgctggctcggaagttcttcacactgtacaagctgtgcgaagaacagctgagtaaacaggtgcactacgacttcggcctgaggaacatcctgagcgtgctgagaactctgggagccgctaagcgggccaaccccatggataccgagagcacaatcgtgatgcgggtgctgcgggacatgaacctgtccaagctgatcgatgaggacgagcccctgtttctgtctctgatcgaggatctgtttcccaacattctgctggataaggccggctaccccgaactggaagctgctatcagcagacaggtggaagaggctggcctgatcaaccaccccccctggaaactgaaagtgatccagctgttcgagacacagcgcgtgcggcacggcatgatgacactgggacctagcggagccggcaagaccacctgtatccacacactgatgcgggccatgaccgattgcggcaagccccaccgcgagatgcggatgaaccccaaggccattaccgcccctcagatgttcggcagactggacgtggccaccaacgactggaccgacggcatcttcagcaccctgtggcgcaagaccctgcgggccaagaagggcgagcacatctggatcatcctggacggccccgtggacgccatctggattgagaacctgaacagcgtgctggacgacaacaagacactgaccctggccaacggcgaccggatccccatggcccccaactgcaagatcatcttcgagccccacaacatcgacaacgccagccctgccaccgtgtccagaaacggcatggtgttcatgagcagcagcatcctggattggagccctatcctggaaggcttcctgaagaagcggagcccccaggaagccgagatcctgagacagctgtacaccgagagcttccccgacctgtaccggttctgcatccagaatctggagtacaagatggaagtgctggaagcctttgtgatcacccagagcatcaacatgctgcagggcctgatccccctgaaagaacagggcggagaagtgtcccaggcccacctgggcagactgttcgtgtttgccctgctgtggagcgctggcgccgctctggaactggatggaaggcggagactggaactgtggctgcggagcagacctaccggcaccctggaactgcctccaccagctggacctggcgacaccgccttcgattactacgtggcccctgacggcacctggacccactggaatacccggacccaggaatacctgtaccccagcgacaccacccccgagtacggctctatcctggtgcccaacgtggacaacgtgcggaccgacttcctgatccagacaatcgccaagcagggaaaggccgtgctgctgatcggcgagcagggcacagccaagaccgtgatcatcaagggctttatgtctaagtacgaccccgagtgccacatgatcaagagcctgaacttcagctccgccaccaccccactgatgttccagcggaccatcgagagctatgtggacaagcggatgggcaccacctacggccctccagccggcaagaaaatgaccgtgttcatcgacgacgtgaacatgcccatcatcaacgagtggggcgaccaagtgaccaacgagatcgtgcggcagctgatggaacagaacggcttctacaacctggaaaagcccggcgagttcacctctatcgtggacatccagtttctggccgccatgatccaccctggcggcggaagaaacgacatcccccagcggctgaagcggcagttcagcatcttcaactgcaccctgcccagcgaggccagcgtggacaagatctttggcgtgatcggcgtgggccactactgcacccagagaggcttcagcgaggaagtgcgggacagcgtgaccaagctggtgcctctgacaagacggctgtggcagatgaccaagatcaagatgctgcccacccccgccaagttccactacgtgttcaacctgcgggacctgagcagagtgtggcagggaatgctgaacaccaccagcgaagtgatcaaagagcccaacgacctgctgaagctgtggaagcacgagtgcaagagagtgatcgccgaccggttcaccgtgtctagcgacgtgacatggttcgacaaggccctggtgtccctggtggaagaggaattcggcgaagagaagaaactgctggtggactgcggcatcgatacctacttcgtggacttcctgcgcgacgcccctgaagccgctggcgagacaagtgaagaggccgacgccgagacacccaagatctacgagcccatcgagtccttcagccatctgaaagaaaggctgaatatgttcctgcagctgtataacgagtccatccggggagccggcatggatatggtgttctttgccgacgccatggtgcacctcgtgaagatcagcagagtgatccggaccccccagggcaacgctctgctcgtgggagtgggaggctctggcaagcagagcctgaccagactggccagctttatcgccggctacgtgtccttccagatcaccctgacccggtcctacaacaccagcaacctgatggaagatctgaaggtgctgtaccggacagccggccagcaggggaagggcatcaccttcatcttcaccgacaatgagatcaaggacgagtctttcctggagtatatgaacaatgtgctgagcagcggcgaggtgtccaacctgttcgcccgggacgagatcgacgagattaacagcgacctggcctccgtgatgaagaaagaattcccccggtgcctgcccacaaacgagaacctgcacgactacttcatgtccagagtgcggcagaatctgcacatcgtgctgtgcttcagccccgtgggcgagaagttcagaaaccgggccctgaagttccccgccctgatcagcggctgcaccatcgactggttcagccggtggcctaaggatgccctggtggccgtgtccgagcactttctgaccagctacgacatcgactgcagcctggaaatcaagaaagaggtggtgcagtgcatgggcagcttccaggacggcgtggccgagaaatgcgtggactacttccagcggttccggcggagcacccacgtgacccctaagagctacctgagcttcatccagggctacaagttcatctacggcgagaagcacgtggaagtgcgcacactggccaaccggatgaacaccggcctggaaaaactgaaagaggcctccgagagcgtggccgccctgagcaaagaactggaagccaaagaaaaagaactgcaggtggccaacgataaggccgacatggtgctgaaagaagtgaccatgaaggcccaggccgccgagaaagtgaaagccgaggtgcagaaagtgaaggaccgggcccaggccatcgtggactccatcagcaaggacaaggccattgccgaggaaaagctggaagcagccaagcccgccctggaagaggcagaagctgctctgcagaccatccggccctccgatattgccacagtgcggaccctgggaaggccccctcacctgatcatgcggatcatggactgtgtgctgctgctgttccagagaaaggtgtccgccgtgaagatcgacctggaaaaatcctgcaccatgcctagctggcaggaatccctgaagctgatgaccgccggcaacttcctgcagaacctgcagcagttccccaaggacaccatcaatgaggaagtgatcgagttcctgagcccctacttcgagatgcccgactacaatatcgaaaccgccaaacgcgtgtgcggcaacgtggccggactgtgctcttggaccaaggctatggctagcttctttagcattaacaaagaggtgctgcctctgaaggccaacctggtggtgcaggaaaaccggcatctgctggccatgcaggacctgcagaaagcccaggccgagctggacgataagcaggctgagctggatgtggtgcaggccgagtacgagcaggccatgaccgagaagcagaccctgctggaagatgcagagcggtgcagacacaagatgcagaccgccagcaccctgatctctggactggccggcgaaaaagagcggtggaccgagcagtcccaggaattcgccgcccagaccaagcggctcgtgggagatgtgctgctggccaccgcctttctgagctacagcggccccttcaatcaggaattcagggacctgctgctgaacgactggcggaaagagatgaaggccagaaagatccccttcggcaagaatctgaacctgagcgagatgctgatcgacgcccccaccatctccgagtggaatctgcagggactgcccaacgatgacctgtccatccagaacggaatcatcgtgaccaaagcctccagataccccctgctgattgacccccagacacagggcaagatttggatcaagaacaaagagagccggaacgagctgcagatcaccagcctgaaccacaagtacttccggaaccacctggaagatagcctgagcctgggcaggccactgctgatcgaggatgtgggcgaggaactggacccagccctggataacgtgctggaacggaacttcatcaagaccggctccaccttcaaagtgaaagtgggcgacaaagaagtggacgtgctggatggcttccggctgtacatcaccaccaagctgcctaaccccgcctacacccctgagatcagcgcccggaccagcatcatcgacttcaccgtgacaatgaagggactggaagatcagctgctgggacgcgtgatcctgacagagaagcaggaactggaaaaagaacggacccatctgatggaagatgtgaccgccaacaagcggcggatgaaggaactggaagataacctgctgtacaggctgaccagcacccagggcagtctggtggaagatgagagcctgatcgtggtgctgtccaacaccaagcggaccgcagaggaagtgacccagaagctggaaatcagcgccgagacagaggtgcagatcaacagcgccagagaagagtaccggcctgtggccacccggggatccatcctgtactttctgatcaccgagatgcggctcgtgaacgagatgtaccagaccagcctgcggcagttcctgggcctgttcgatctgtccctggccagaagcgtgaagtcccccatcaccagcaagagaatcgccaacatcatcgagcacatgacctacgaggtgtacaaatacgccgccagaggcctgtacgaggaacacaagtttctgttcacactgctgctgaccctgaagatcgatatccagcggaacagagtgaagcacgaagagtttctgacactgatcaaggggggagcctccctggacctgaaggcctgtcctcccaagcccagcaagtggatcctggacatcacctggctgaatctggtggaactgagcaagctgagacagttctccgatgtgctggaccagatcagccgcaacgagaagatgtggaagatttggtttgacaaagagaaccccgaggaagaacccctgcctaacgcctacgataagagcctggactgcttccggcggctgctgctgattagaagctggtgtcccgaccggacaatcgcccaggcccgcaagtacatcgtggatagcatgggagagaagtacgccgagggcgtgatcctggacctggaaaagacctgggaggaaagcgaccccagaacccccctgatctgcctgctgagcatgggctccgaccccaccgacagcattatcgccctgggcaagagactgaagattgagacaagatacgtgtccatgggccagggccaggaagtgcacgctagaaagctgctgcagcagactatggccaatggcggctgggccctgctgcagaattgtcacctggggctggacttcatggacgaactgatggacatcatcattgagacagagctggtgcacgacgccttcagactgtggatgaccaccgaggcccataagcagtttcccattaccctgctgcagatgagcatcaagttcgccaacgacccccctcagggactgagagccggcctgaagagaacctactccggcgtgtcacaggatctgctggacgtgtcctctggcagccagtggaagcctatgctgtacgccgtggcattcctgcacagcaccgtgcaggaacggcggaagtttggcgccctgggatggaacatcccctacgagtttaaccaggccgacttcaacgccactgtgcagtttatccagaaccatctggacgacatggacgtgaagaaaggggtgtcctggacaaccatccggtacatgatcggagagatccagtacggcggcagagtgaccgacgactacgacaagaggctgctgaataccttcgccaaagtgtggttctccgagaacatgtttggccccgacttcagcttttaccagggctataacatccccaagtgctccaccgtggataactacctgcagtacatccagagcctgcccgcctacgacagccctgaggtgttcggactgcaccccaacgccgatatcacctaccagagcaaactggccaaggatgtgctggataccatcctgggcatccagcccaaggataccagtggcggaggcgacgaaacccgggaagcagtggtggctagactggccgacgacatgctggaaaagctgccccccgactacgtgccctttgaagtgaaagaacgcctgcagaagatgggccccttccagcctatgaacatcttcctgaggcaggaaatcgaccggatgcagcgggtgctgtctctcgtgcggagcacactgaccgagctgaaactggctatcgacggcaccatcatcatgagcgagaatctgcgggatgcactggactgcatgttcgacgccagaatccccgcatggtggaaaaaggccagctggatcagctctaccctgggcttctggttcaccgaactgatcgagagaaacagccagtttaccagctgggtgttcaacggcagacctcactgcttctggatgaccggcttcttcaatccacaaggctttctgacagcaatgcgccaggaaatcaccagagccaacaagggctgggctctggacaatatggtgctgtgtaacgaagtgactaagtggatgaaggacgacatcagcgcccctcccacagagggcgtgtacgtgtacggcctgtacctggaaggcgccggatgggacaagagaaacatgaagctgatcgagagcaagcccaaggtgctgttcgagctgatgcccgtgatcaggatctatgccgagaacaacaccctgagggacccccggttctacagctgccccatctacaagaaacccgtgcgcaccgacctgaactatatcgccgccgtggacctgaggacagcccagacacctgagcattgggtgctgagaggcgtggcactgctgtgcgacgtgaagtga

SEQ ID NO: 19 - RNA, 10 nt, synthetic construct
  misc_feature 1..10: note = Description of Artificial Sequence: Synthetic oligonucleotide
  source 1..10: mol_type = other RNA
gccrccatgg

SEQ ID NO: 20 - DNA, 11 bp, synthetic construct
  misc_feature 1..11: note = Description of Artificial Sequence: Synthetic oligonucleotide
  source 1..11: mol_type = other DNA
gaattctgcag